European Patent Specification EP 4 294 939 B1, published November 12, 2025. Title: METHODS FOR IDENTIFICATION AND TREATMENT OF BLEEDING IN ANIMALS. Applicant: Washington State University. The sequence listing filed with the application follows.

SEQUENCE LISTING (16 sequences)

SEQ ID NO: 1 - DNA, 9721 bp, Canis lupus
cctgcctcgcctgcccacccctcaccacagtgtttgtgccttgaactgaggaggcagcccctgagcccagaactcttatggtccaacaccccgagagaaggggtgagaataatctctgcatctcaggtctcccaggaaatgggaagacccaggcatcccaggaccctcacattctggagcagagatgagatctgagcctgtgcccctactgcctcctcattatttgcaatagatgtaaatatgaccaataaatcctttggaagagccatggacctgagtgatgcttttctcgacgatggcatcagggtggggaagaatcgagactcagtagcttccagggcagtgaagacagagtgagaagtagggcaggagagtgggagacagcctaatcgctgcttttgggcaccacagggtacagggcttctggatcaagcagcccccctcagaggaggctcagccctggcgggatgttaaggaggcattgctcctgctgagggaggatgctgcctggtactgtgaccctctctcctctccccactccttctagatccagtctaaaaggcagccaatcaggatcctggcttgtaaggtttgaggatgggcatcttgagctccccacataagctcctacagcttccccttcctccccctcatgataggggagaggaaagaacattggaagtgagaagctggatgtgactcgagcctagctctgtccttgggcacgtcacctaccctctctgactccagtaaagtagagataaaccccccccacctcatggggttgctggaaggcccctgtccttcctggatctgtcgtacagatgaggacatcttccttaactttcccgaatctcctttctccaggcgtgggtgggacccaaatccacagggctccaggtggctatctcaggattagatgccctggtgggaatggggtttccggccccagtatcaatgtttaaccggatgtgctggtcaatatttaccagaagagaaatctgaacaatctgaacaggggttggctgagagcaaaggtcctggtgggaggggagggctcagatgggctggctggagcctgagcaaagtgtggggagcaccacagtggggccagagggacattgtgtgcagcagcaaggagcctacagaggtacgaggggaggggtggcttggcctgctctttgggccagataggaggtaagagctgcccacccggctgaaggggtctggggtgaatttattcagaaggcctctcatttcccagcctcctggggtgatgaggagccaaggtgggggttctggcaggagtctctctgggacttgaaaaactggaggtcttttcttgtcaggaggattcaaaacccccattagagattagggccctggccaagggtccttgtgtgtgatggaggtggggccaggggtgatagaggatcccctggaaggactggccctgagatgggggcggggttggagtgtatgggacctgctctgaggccagactaagacctgcccatccccacctgctggctgggcttcccggagccgacctggacagagtcgggcacaaggcctatgtttcccgtaagtccaaaggtggctctatccagaaccattcattgggctctgtggctaggtcaacaacaaggctctccggcccatcccaccaaacctgccgagacctcagggattcacaggcctgtctacccttgtggtcaagaccagaccaagaaaaggtgggccattgggcagcaggttgggtaggagctctgggtaaggagccctaggacacaggaggcttcagggcaggcttcccagaagaggggccttgggctaggctgacaacagccataccactgagtgccaggcagcgtaaccagggttcacaaagactgtctcattttggtcctcacagtataccgtgggaggaggtagggacttttgctaccattttacaagaaaaggcaaagcccagggagctatctgagggcctctgggaagaggcagagtctggattccaatcgatgttggactcacaatgccaggcctcgaagaatgaggacttctttcattttgattatttcccctatgaaccaaaacattttcagtgcatgacatgtggaaaactggaaaattcaaaagggctgaaaaggattcagggggatatcccgccccacggagatgagaaacagggctcgtgggtgttgggagtgctggcggtggtggctggattgacctgccctcccaggcagcgtgtgggtgggcccccgggagtggggtcggtggggacggggacgcaggctgcctgtccccgcacaggaacatggcgctgctccgggggctcctggtgatcagcttgtcctgcctccaaggctccggcgcggtggtgagcctgggcctccctgggggggagggggctgagtcaagggagcgtttggctctgaagagctccctctcttcccctcatccttttctcgacagttccctcctgccagcgccatggagcccttggaccagcaggtactcgggagtgagaggcaggagggggaggaaagccccgcgggcctaacctgtggttggcgcagggagtgggccgacccgtgggaagggtcacgctccatttgcttcctcccttcttcagctaatgggcgggcagacccaagagaagctgcccccgctcaccctcctcaagttgggcaaccaggtacaaccaggtggggctggggaagagtgggcggggtccgagggaggagggccaatcagcggggccacgactcagagggtgggaggggccagaggaaaggaccaggtccttgtactgtcattgtccatgtgactgtccctctcttgccaggactattcttgggcaggggggctgtggaagggatcttcaacacagagcggactccttgaccctcttgacccctgatctgtctgtaggagtccagtggccatattggcctgaagaaggccccaagagactgcaggggagccccaaccccagagcagacccgcagattggcccaggccatgatggccttcaccacagacctgttctccctggtggcccaaaggtccaccagccccaacctaatcctgtcgcctctgagtgtggccctggcactgtctcacctggcactaggtactgtggcatcacctgtccagaccagcagagctggaggccagtgggaactcactactccagagtttactagtgggtgcctcctgcatcagagtcacttggatgtttggtaaaaatgcagattcctaggtacacctccagtctctgtgaatcagattcccagggattgggcctaaggatatgcttctggtgatttttacataagcctttgataactacaatgtctccaccggactggagactctcattgtgggaaaccgaggtccagagagggaatacgacttggatcgagtgaggtgacccagactgccagcagcagagacaaaagtagaacttggggagtattgtcaccccaatcagtttagtggatacggggggagaatgtgtggtgtcgtggccatgctcacgatggggatttaacagagcctggagtggccagtaggggtgggaaagtgccactggcctgggccaaagcccatgtggtcccctccaggtgctcagaaccagacgctgcggaggttagagcaggtgctgcatgcagactctgggccctgcctcccccacctgctgagccgcctttgccaggacctgggccctggggcattccgattggctgctagaatgtacctgcagaaaggtaggtgctggtggcttggagctccctaggttgtgccctggagtggacaggagtgatggagatgggtttggccttaggcagccagtcagagcattggtggctctggagctcaagcccttaggaacagcttgtggccttttctgtgtaggatttcccatcaaagaggacttcctgaaacaatcagaacagctctttggtgccaagcccatgagcctgaccggaaggaaaggggatgatctgctaaacatcaaccaatgggtgaaggaggccacagaggggaagattgaggatttcctctcagagctgccagatgacacagtgttgcttctgctcaatgccatccacttccagggtgcgttccccctcttctctggccctctacccctgtggcccctattcctgccttgtaggctgaactgggctgcaaaacctttgttctgagggtctctctttctcctcagggctgggtcaggaggcagggagctttctaggttgtggcttgggggagggtaggaaacaggtaatggtgtgccagtgaggggcctcaggaactggatgagagaaccctaggaggaaactgagtctgaaaggattgagggtggggttgggggtgctcctgggagcatgacaggacataggaagaatgcaagcccagatttcaaaaatgctgcagggaagaaacctcagatcaactgggaatcaactggcacagtgccccttgggcttttgacttctactttttgtcccttgaatgggttctgggtgggatggagaagagactagtggtgtggaacccacccctgtcccagtctacgtgacccctgccctctgctggatataggtttctggaggagcaagtttgatccaagcctcacccagagagacagtttccacctgaacgagcagttcacggtgccagtggacatgatgcacgcccgcacgtaccccctgcgctggttcctgctggagcagcctgagatacaggtcacccttgactgcccaggctgggcctggctgctgggaggtggggcagggggggcaggctgtgggacaggtacaggggtggaggggggtgtgccccacctcccttgcagtcttgtccctgagacaggtggctctggaaggtcacattatgccctgatccagagggactgaggttccaggctctttgaagttcaagaatttgacaaaactatattaggcatttgccaccagaacacactagcacaagggagaccaagtccctgctctcaggaggaaagacacacacagtacacggacagacataaatcatggaataatttcacatagtataactgctatgaaggaaaaaaataaagtgatcaattagtgacaggggaaggtattttattttatttatttttttaaagaagttctttttttaattttttttatttatttatgatagtcacagagagagagagagagagagagagagagaggcagagacataggcagagggaaaagcaggctccatgcaccgggagcccgacgtgggatttgatcccaggtctcgaggatcacgccctgggccaaaggcaggcactaaaccgctgtgccacccagggatccctggggaaggtattttagataaagtggtcagggagcagtctatgaggaggggcctcaagtggagaaccagatgatttttggtcagaggggtttattacaagggcccatggattggtcaggctgcaaaggagccacccaacagctacagagccactcaggcctcagcatcctcgagcctgggagacgtgatctgactgtcacagtgctccttggaagggaggatctggttgcaatggatttgtcagtaacctgctggaacattctgattggatagagtactatgccaagcggtctcaggtgaggcctcccttgcttctagcctaaatgtggtcctcttggcttgagcatggacccctgggcccatccactgtggcagagatggcaatgttggttagtttcccaaggcagcatgccacaggcctcagcgactcctgagaggggctgtgggggcaaggcagacccttggagcagcgtccagcttctctcgctttcaccccgacgggcagactgtcttgttcacctccccacctgttctctttgtgctgctcctgccctccaggctgtgtcctgcccactctttcttcacccatcctctctgtccctggcctctgccctcctcttcctcacacactctgcaggctgacccagacagccagatgtggtgttccccaccacccccgccacccccaaggttcctgctccctggctgctctgcctagagactaagaagtctcacttgccagggatcatcatgcccagtgcttctcatactcaagtagctgcagaaaccccattcacatgacatcttacctcagatcacagtatcatatacaccctaggtgaaggtgtgggggggagaaccacctgttgcagtggctcctctgtaggacctagggtggtttgaaaacgaacaacccagtccattgtacacgtggagacactgagaggcagagctggttacagacgaagagagggaaagtcccccctttattgagcactgcccatgtgctgatactccactagaagctttaaaagggtctctctctctcttttttttctctctctcacatgtcaacctacaatgtgggcaggcagtgttactccacttcacaggtgaggaagtgggggctcagggaggctgaacacacacctgagaacaatggactggaactcctgctccatctgtctcagaagcctatgctggcccagaccccagctggtatgggcaccttctggccctcaccgctgtctcctttctttctctgtaggtggctcatttcccctttaagaacaacatgagctttgtggtcattatgcccacccactttgagtggaacgtgtcccaggtgctggccaacctgagctgggacatcctgcaccagcccttactgcgagagaaacccaccaaggtccggctgcctaagctgcacctgaactaccagctggacttggtggccaccctcagccggctgggtaaggaagggtgaggcttgggtaaggacagtcccctaggccaggctaggcagagcaagtgaggaacaaagccccagctggcagtaggtccgagtcagagcagccttgtgtcctggccttctctggggctttgggaggtgagggcttcctaggaccccccagatcctccgtcccgggatgggctggggtggcccagggaatgaggatctgctccatccaagactgaacattgtgaagaatcttgggtagagagcctgcgtggcacgtgagccttgctggctgtcctgcaaggggcactgtactaggtacaaggggctcaggcagatgcggaatcaggtacttactatacagcttaggtgatgagtcagagggcttctctccagttcactggagaagggcacccggccggaccttggggcaggggatccagaaagtctccttggaggaagtgacctttaagccaataactggaggttaagtgagagttccccaaggatctgtgggttggaggtgttcccggccagaatgctagccaccgtcccaggcaggtcccggcagcctgcggggcagaaggcagctctgaccggcagtctcttgccctgggcaggcctgcaggagctgttccaggccccagacctgcgcgggatctccgaccagcgcctggtggtgaccagcgtgcagcaccagtctgctctggagctcagtgaggctggtgtggaggcggccgcggccacgggcacggccatgtcccgaatgtctctctcctccttcagcgtcaaccgccccttcctcttcttcatcctcgaggacacaacaagcctgcccctgtttgtgggcagtgtgaagaaccccaaccctagtgcgccatgggagcgcaaggagcagcaggattcccccgatgacagggactacttccagaaccggaaagcctttccccgcggagacaagcccttcgggcctgacttgaaacttgcgcctccctcagaggaggattacccccaacttcatagccccaagtgagaggccagctgccagcatcccgagtccctgctggagcaacctctcaactcttgtgactctttccagacagcattgtgggaggagggcagggacctgggtggggagtctgggagcccagagggagccactctctcaagtctcctcctctcagggattttggggttgggggggccacaggacggggcggacctcaggtaatcaagggccttcatcccacatctcttcttccaaaagcgactcagaggctgtcctttgggggacttgggcagaagggcagctggagaagctggagatccacttttgtcaggaaggtagttcccgtgttggctgtggcacttccacgtttgtttacgggggggggggggtgttgggggggcaggggggcaggagggatggaataccttggctggggagaggacagtaggccctgggggtgtggagcctgggcctgctctatgggcggggcctagaattccacaaactgcttctgccacacttgctggaggccctccagcccccatcccccaacccgccccccacaccctgtcacttcagcctccccactgctcctaggagataccagcattgccaggactcttcttccctgtctctcctcttcttcctctgcccaggtgtctcaggtgggaggtgtgtgtgtggggaatagttaactccctaaggctcttttgtaaagtttttgtagtgatttttatgccacctgaataaagaatgaatgaccctggctgttttgatgtcactctgctgggcatgggctggagcaagggggctgagggaggcaggagggccctggcggcactgagcctcacgctgggccctgacagcacacagcaggcggccctctctgccacgtttgtcccctggccacccgccagctcttccccggcgcagtcccctctgaccttgccagccctctctgcggccagctccatgccagccgggctccactctctccagaggcctcaagcagccattaacaagggtggctcagaatagcgctggcctcccagtttggagaaaactggcaattagggagcttgtggagtttctaattacatgtcagtccttctggcaggggcaggcgcccgtcagccagggacaggctgcagggagcactggttccagctggacgctgtcatgcctgaggatctgggggaaacagttgggcccaccttggcccggggccgtgggtggtatgcagggccacgtgcgtgggcccttatctgtgggtacagggtgtccctgtggccgtggccacctgaagccccgaagtgcagtggtcaagagcaagtgcccagggtggactctggcttcctacaaaccagcaatgtggggagacaggtgaaatcgatgatgaggcagagggtggttggttagagccgtggtgagaaatagagcagggaaggcctccctgagaaggtggtacgggagcagagacttgaggcaggtgaaggcaggcatgatataaataaccagggcagagttcctgggtggaagcatgctcagaaggttcaggatggggatccctgggtggcgcagcggtttggcgcttgcctttggcccagggcgcgatcctggagacccgggatcaaatcccacgtcgggctcctggtgcatggagcccgcttctccctcaacctgtgtctctgcctctctctctctctctgtgactatcataaaaaaaaaaaaaaattagaaggttcaggatgaacagggggtccgtggagctagaggggaggggtaggagtgagtcagaggggaacatgtactagtgctttagggccactgtaaagactgttgtttttatcttaggagtaagaagtaattggatagttaaa

SEQ ID NO: 2 - DNA, 1668 bp, Artificial Sequence
  Synthetic gene construct
atgggctggctggagcctgagcaaagtgtggggagcaccacagtggggccagagggacattgtgtgcagcagcaaggagcctacagaggtcaacaacaaggctctccggcccatcccaccaaacctgccgagacctcagggattcacaggcctgtctacccttgtggtcaagaccagaccaagaaaaggaacatggcgctgctccgggggctcctggtgatcagcttgtcctgcctccaaggctccggcgcggtgttccctcctgccagcgccatggagcccttggaccagcagctaatgggcgggcagacccaagagaagctgcccccgctcaccctcctcaagttgggcaaccaggagtccagtggccatattggcctgaagaaggccccaagagactgcaggggagccccaaccccagagcagacccgcagattggcccaggccatgatggccttcaccacagacctgttctccctggtggcccaaaggtccaccagccccaacctaatcctgtcgcctctgagtgtggccctggcactgtctcacctggcactaggtgctcagaaccagacgctgcggaggttagagcaggtgctgcatgcagactctgggccctgcctcccccacctgctgagccgcctttgccaggacctgggccctggggcattccgattggctgctagaatgtacctgcagaaaggatttcccatcaaagaggacttcctgaaacaatcagaacagctctttggtgccaagcccatgagcctgaccggaaggaaaggggatgatctgctaaacatcaaccaatgggtgaaggaggccacagaggggaagattgaggatttcctctcagagctgccagatgacacagtgttgcttctgctcaatgccatccacttccagggtttctggaggagcaagtttgatccaagcctcacccagagagacagtttccacctgaacgagcagttcacggtgccagtggacatgatgcacgcccgcacgtaccccctgcgctggttcctgctggagcagcctgagatacaggtggctcatttcccctttaagaacaacatgagctttgtggtcattatgcccacccactttgagtggaacgtgtcccaggtgctggccaacctgagctgggacatcctgcaccagcccttactgcgagagaaacccaccaaggtccggctgcctaagctgcacctgaactaccagctggacttggtggccaccctcagccggctgggcctgcaggagctgttccaggccccagacctgcgcgggatctccgaccagcgcctggtggtgaccagcgtgcagcaccagtctgctctggagctcagtgaggctggtgtggaggcggccgcggccacgggcacggccatgtcccgaatgtctctctcctccttcagcgtcaaccgccccttcctcttcttcatcctcgaggacacaacaagcctgcccctgtttgtgggcagtgtgaagaaccccaaccctagtgcgccatgggagcgcaaggagcagcaggattcccccgatgacagggactacttccagaaccggaaagcctttccccgcggagacaagcccttcgggcctgacttgaaacttgcgcctccctcagaggaggattacccccaacttcatagccccaagtga

SEQ ID NO: 3 - protein, 555 aa, Canis lupus
MGWLEPEQSVGSTTVGPEGHCVQQQGAYRGQQQGSPAHPTKPAETSGIHRPVYPCGQDQTKKRNMALLRGLLVISLSCLQGSGAVFPPASAMEPLDQQLMGGQTQEKLPPLTLLKLGNQESSGHIGLKKAPRDCRGAPTPEQTRRLAQAMMAFTTDLFSLVAQRSTSPNLILSPLSVALALSHLALGAQNQTLRRLEQVLHADSGPCLPHLLSRLCQDLGPGAFRLAARMYLQKGFPIKEDFLKQSEQLFGAKPMSLTGRKGDDLLNINQWVKEATEGKIEDFLSELPDDTVLLLLNAIHFQGFWRSKFDPSLTQRDSFHLNEQFTVPVDMMHARTYPLRWFLLEQPEIQVAHFPFKNNMSFVVIMPTHFEWNVSQVLANLSWDILHQPLLREKPTKVRLPKLHLNYQLDLVATLSRLGLQELFQAPDLRGISDQRLVVTSVQHQSALELSEAGVEAAAATGTAMSRMSLSSFSVNRPFLFFILEDTTSLPLFVGSVKNPNPSAPWERKEQQDSPDDRDYFQNRKAFPRGDKPFGPDLKLAPPSEEDYPQLHSPK

SEQ ID NO: 4 - DNA, 9721 bp, Canis lupus
cctgcctcgcctgcccacccctcaccacagtgtttgtgccttgaactgaggaggcagcccctgagcccagaactcttatggtccaacaccccgagagaaggggtgagaataatctctgcatctcaggtctcccaggaaatgggaagacccaggcatcccaggaccctcacattctggagcagagatgagatctgagcctgtgcccctactgcctcctcattatttgcaatagatgtaaatatgaccaataaatcctttggaagagccatggacctgagtgatgcttttctcgacgatggcatcagggtggggaagaatcgagactcagtagcttccagggcagtgaagacagagtgagaagtagggcaggagagtgggagacagcctaatcgctgcttttgggcaccacagggtacagggcttctggatcaagcagcccccctcagaggaggctcagccctggcgggatgttaaggaggcattgctcctgctgagggaggatgctgcctggtactgtgaccctctctcctctccccactccttctagatccagtctaaaaggcagccaatcaggatcctggcttgtaaggtttgaggatgggcatcttgagctccccacataagctcctacagcttccccttcctccccctcatgataggggagaggaaagaacattggaagtgagaagctggatgtgactcgagcctagctctgtccttgggcacgtcacctaccctctctgactccagtaaagtagagataaaccccccccacctcatggggttgctggaaggcccctgtccttcctggatctgtcgtacagatgaggacatcttccttaactttcccgaatctcctttctccaggcgtgggtgggacccaaatccacagggctccaggtggctatctcaggattagatgccctggtgggaatggggtttccggccccagtatcaatgtttaaccggatgtgctggtcaatatttaccagaagagaaatctgaacaatctgaacaggggttggctgagagcaaaggtcctggtgggaggggagggctcagatgggctggctggagcctgagcaaagtgtggggagcaccacagtggggccagagggacattgtgtgcagcagcaaggagcctacagaggtacgaggggaggggtggcttggcctgctctttgggccagataggaggtaagagctgcccacccggctgaaggggtctggggtgaatttattcagaaggcctctcatttcccagcctcctggggtgatgaggagccaaggtgggggttctggcaggagtctctctgggacttgaaaaactggaggtcttttcttgtcaggaggattcaaaacccccattagagattagggccctggccaagggtccttgtgtgtgatggaggtggggccaggggtgatagaggatcccctggaaggactggccctgagatgggggcggggttggagtgtatgggacctgctctgaggccagactaagacctgcccatccccacctgctggctgggcttcccggagccgacctggacagagtcgggcacaaggcctatgtttcccgtaagtccaaaggtggctctatccagaaccattcattgggctctgtggctaggtcaacaacaaggctctccggcccatcccaccaaacctgccgagacctcagggattcacaggcctgtctacccttgtggtcaagaccagaccaagaaaaggtgggccattgggcagcaggttgggtaggagctctgggtaaggagccctaggacacaggaggcttcagggcaggcttcccagaagaggggccttgggctaggctgacaacagccataccactgagtgccaggcagcgtaaccagggttcacaaagactgtctcattttggtcctcacagtataccgtgggaggaggtagggacttttgctaccattttacaagaaaaggcaaagcccagggagctatctgagggcctctgggaagaggcagagtctggattccaatcgatgttggactcacaatgccaggcctcgaagaatgaggacttctttcattttgattatttcccctatgaaccaaaacattttcagtgcatgacatgtggaaaactggaaaattcaaaagggctgaaaaggattcagggggatatcccgccccacggagatgagaaacagggctcgtgggtgttgggagtgctggcggtggtggctggattgacctgccctcccaggcagcgtgtgggtgggcccccgggagtggggtcggtggggacggggacgcaggctgcctgtccccgcacaggaacatggcgctgctccgggggctcctggtgatcagcttgtcctgcctccaaggctccggcgcggtggtgagcctgggcctccctgggggggagggggctgagtcaagggagcgtttggctctgaagagctccctctcttcccctcatccttttctcgacagttccctcctgccagcgccatggagcccttggaccagcaggtactcgggagtgagaggcaggagggggaggaaagccccgcgggcctaacctgtggttggcgcagggagtgggccgacccgtgggaagggtcacgctccatttgcttcctcccttcttcagctaatgggcgggcagacccaagagaagctgcccccgctcaccctcctcaagttgggcaaccaggtacaaccaggtggggctggggaagagtgggcggggtccgagggaggagggccaatcagcggggccacgactcagagggtgggaggggccagaggaaaggaccaggtccttgtactgtcattgtccatgtgactgtccctctcttgccaggactattcttgggcaggggggctgtggaagggatcttcaacacagagcggactccttgaccctcttgacccctgatctgtctgtaggagtccagtggccatattggcctgaagaaggccccaagagactgcaggggagccccaaccccagagcagacccgcagattggcccaggccatgatggccttcaccacagacctgttctccctggtggcccaaaggtccaccagccccaacctaatcctgtcgcctctgagtgtggccctggcactgtctcacctggcactaggtactgtggcatcacctgtccagaccagcagagctggaggccagtgggaactcactactccagagtttactagtgggtgcctcctgcatcagagtcacttggatgtttggtaaaaatgcagattcctaggtacacctccagtctctgtgaatcagattcccagggattgggcctaaggatatgcttctggtgatttttacataagcctttgataactacaatgtctccaccggactggagactctcattgtgggaaaccgaggtccagagagggaatacgacttggatcgagtgaggtgacccagactgccagcagcagagacaaaagtagaacttggggagtattgtcaccccaatcagtttagtggatacggggggagaatgtgtggtgtcgtggccatgctcacgatggggatttaacagagcctggagtggccagtaggggtgggaaagtgccactggcctgggccaaagcccatgtggtcccctccaggtgctcagaaccagacgctgcggaggttagagcaggtgctgcatgtagactctgggccctgcctcccccacctgctgagccgcctttgccaggacctgggccctggggcattccgattggctgctagaatgtacctgcagaaaggtaggtgctggtggcttggagctccctaggttgtgccctggagtggacaggagtgatggagatgggtttggccttaggcagccagtcagagcattggtggctctggagctcaagcccttaggaacagcttgtggccttttctgtgtaggatttcccatcaaagaggacttcctgaaacaatcagaacagctctttggtgccaagcccatgagcctgaccggaaggaaaggggatgatctgctaaacatcaaccaatgggtgaaggaggccacagaggggaagattgaggatttcctctcagagctgccagatgacacagtgttgcttctgctcaatgccatccacttccagggtgcgttccccctcttctctggccctctacccctgtggcccctattcctgccttgtaggctgaactgggctgcaaaacctttgttctgagggtctctctttctcctcagggctgggtcaggaggcagggagctttctaggttgtggcttgggggagggtaggaaacaggtaatggtgtgccagtgaggggcctcaggaactggatgagagaaccctaggaggaaactgagtctgaaaggattgagggtggggttgggggtgctcctgggagcatgacaggacataggaagaatgcaagcccagatttcaaaaatgctgcagggaagaaacctcagatcaactgggaatcaactggcacagtgccccttgggcttttgacttctactttttgtcccttgaatgggttctgggtgggatggagaagagactagtggtgtggaacccacccctgtcccagtctacgtgacccctgccctctgctggatataggtttctggaggagcaagtttgatccaagcctcacccagagagacagtttccacctgaacgagcagttcacggtgccagtggacatgatgcacgcccgcacgtaccccctgcgctggttcctgctggagcagcctgagatacaggtcacccttgactgcccaggctgggcctggctgctgggaggtggggcagggggggcaggctgtgggacaggtacaggggtggaggggggtgtgccccacctcccttgcagtcttgtccctgagacaggtggctctggaaggtcacattatgccctgatccagagggactgaggttccaggctctttgaagttcaagaatttgacaaaactatattaggcatttgccaccagaacacactagcacaagggagaccaagtccctgctctcaggaggaaagacacacacagtacacggacagacataaatcatggaataatttcacatagtataactgctatgaaggaaaaaaataaagtgatcaattagtgacaggggaaggtattttattttatttatttttttaaagaagttctttttttaattttttttatttatttatgatagtcacagagagagagagagagagagagagagagaggcagagacataggcagagggaaaagcaggctccatgcaccgggagcccgacgtgggatttgatcccaggtctcgaggatcacgccctgggccaaaggcaggcactaaaccgctgtgccacccagggatccctggggaaggtattttagataaagtggtcagggagcagtctatgaggaggggcctcaagtggagaaccagatgatttttggtcagaggggtttattacaagggcccatggattggtcaggctgcaaaggagccacccaacagctacagagccactcaggcctcagcatcctcgagcctgggagacgtgatctgactgtcacagtgctccttggaagggaggatctggttgcaatggatttgtcagtaacctgctggaacattctgattggatagagtactatgccaagcggtctcaggtgaggcctcccttgcttctagcctaaatgtggtcctcttggcttgagcatggacccctgggcccatccactgtggcagagatggcaatgttggttagtttcccaaggcagcatgccacaggcctcagcgactcctgagaggggctgtgggggcaaggcagacccttggagcagcgtccagcttctctcgctttcaccccgacgggcagactgtcttgttcacctccccacctgttctctttgtgctgctcctgccctccaggctgtgtcctgcccactctttcttcacccatcctctctgtccctggcctctgccctcctcttcctcacacactctgcaggctgacccagacagccagatgtggtgttccccaccacccccgccacccccaaggttcctgctccctggctgctctgcctagagactaagaagtctcacttgccagggatcatcatgcccagtgcttctcatactcaagtagctgcagaaaccccattcacatgacatcttacctcagatcacagtatcatatacaccctaggtgaaggtgtgggggggagaaccacctgttgcagtggctcctctgtaggacctagggtggtttgaaaacgaacaacccagtccattgtacacgtggagacactgagaggcagagctggttacagacgaagagagggaaagtcccccctttattgagcactgcccatgtgctgatactccactagaagctttaaaagggtctctctctctcttttttttctctctctcacatgtcaacctacaatgtgggcaggcagtgttactccacttcacaggtgaggaagtgggggctcagggaggctgaacacacacctgagaacaatggactggaactcctgctccatctgtctcagaagcctatgctggcccagaccccagctggtatgggcaccttctggccctcaccgctgtctcctttctttctctgtaggtggctcatttcccctttaagaacaacatgagctttgtggtcattatgcccacccactttgagtggaacgtgtcccaggtgctggccaacctgagctgggacatcctgcaccagcccttactgcgagagaaacccaccaaggtccggctgcctaagctgcacctgaactaccagctggacttggtggccaccctcagccggctgggtaaggaagggtgaggcttgggtaaggacagtcccctaggccaggctaggcagagcaagtgaggaacaaagccccagctggcagtaggtccgagtcagagcagccttgtgtcctggccttctctggggctttgggaggtgagggcttcctaggaccccccagatcctccgtcccgggatgggctggggtggcccagggaatgaggatctgctccatccaagactgaacattgtgaagaatcttgggtagagagcctgcgtggcacgtgagccttgctggctgtcctgcaaggggcactgtactaggtacaaggggctcaggcagatgcggaatcaggtacttactatacagcttaggtgatgagtcagagggcttctctccagttcactggagaagggcacccggccggaccttggggcaggggatccagaaagtctccttggaggaagtgacctttaagccaataactggaggttaagtgagagttccccaaggatctgtgggttggaggtgttcccggccagaatgctagccaccgtcccaggcaggtcccggcagcctgcggggcagaaggcagctctgaccggcagtctcttgccctgggcaggcctgcaggagctgttccaggccccagacctgcgcgggatctccgaccagcgcctggtggtgaccagcgtgcagcaccagtctgctctggagctcagtgaggctggtgtggaggcggccgcggccacgggcacggccatgtcccgaatgtctctctcctccttcagcgtcaaccgccccttcctcttcttcatcctcgaggacacaacaagcctgcccctgtttgtgggcagtgtgaagaaccccaaccctagtgcgccatgggagcgcaaggagcagcaggattcccccgatgacagggactacttccagaaccggaaagcctttccccgcggagacaagcccttcgggcctgacttgaaacttgcgcctccctcagaggaggattacccccaacttcatagccccaagtgagaggccagctgccagcatcccgagtccctgctggagcaacctctcaactcttgtgactctttccagacagcattgtgggaggagggcagggacctgggtggggagtctgggagcccagagggagccactctctcaagtctcctcctctcagggattttggggttgggggggccacaggacggggcggacctcaggtaatcaagggccttcatcccacatctcttcttccaaaagcgactcagaggctgtcctttgggggacttgggcagaagggcagctggagaagctggagatccacttttgtcaggaaggtagttcccgtgttggctgtggcacttccacgtttgtttacgggggggggggggtgttgggggggcaggggggcaggagggatggaataccttggctggggagaggacagtaggccctgggggtgtggagcctgggcctgctctatgggcggggcctagaattccacaaactgcttctgccacacttgctggaggccctccagcccccatcccccaacccgccccccacaccctgtcacttcagcctccccactgctcctaggagataccagcattgccaggactcttcttccctgtctctcctcttcttcctctgcccaggtgtctcaggtgggaggtgtgtgtgtggggaatagttaactccctaaggctcttttgtaaagtttttgtagtgatttttatgccacctgaataaagaatgaatgaccctggctgttttgatgtcactctgctgggcatgggctggagcaagggggctgagggaggcaggagggccctggcggcactgagcctcacgctgggccctgacagcacacagcaggcggccctctctgccacgtttgtcccctggccacccgccagctcttccccggcgcagtcccctctgaccttgccagccctctctgcggccagctccatgccagccgggctccactctctccagaggcctcaagcagccattaacaagggtggctcagaatagcgctggcctcccagtttggagaaaactggcaattagggagcttgtggagtttctaattacatgtcagtccttctggcaggggcaggcgcccgtcagccagggacaggctgcagggagcactggttccagctggacgctgtcatgcctgaggatctgggggaaacagttgggcccaccttggcccggggccgtgggtggtatgcagggccacgtgcgtgggcccttatctgtgggtacagggtgtccctgtggccgtggccacctgaagccccgaagtgcagtggtcaagagcaagtgcccagggtggactctggcttcctacaaaccagcaatgtggggagacaggtgaaatcgatgatgaggcagagggtggttggttagagccgtggtgagaaatagagcagggaaggcctccctgagaaggtggtacgggagcagagacttgaggcaggtgaaggcaggcatgatataaataaccagggcagagttcctgggtggaagcatgctcagaaggttcaggatggggatccctgggtggcgcagcggtttggcgcttgcctttggcccagggcgcgatcctggagacccgggatcaaatcccacgtcgggctcctggtgcatggagcccgcttctccctcaacctgtgtctctgcctctctctctctctctgtgactatcataaaaaaaaaaaaaaattagaaggttcaggatgaacagggggtccgtggagctagaggggaggggtaggagtgagtcagaggggaacatgtactagtgctttagggccactgtaaagactgttgtttttatcttaggagtaagaagtaattggatagttaaa

SEQ ID NO: 5 - DNA, 1668 bp, Artificial Sequence
  Synthetic gene construct
atgggctggctggagcctgagcaaagtgtggggagcaccacagtggggccagagggacattgtgtgcagcagcaaggagcctacagaggtcaacaacaaggctctccggcccatcccaccaaacctgccgagacctcagggattcacaggcctgtctacccttgtggtcaagaccagaccaagaaaaggaacatggcgctgctccgggggctcctggtgatcagcttgtcctgcctccaaggctccggcgcggtgttccctcctgccagcgccatggagcccttggaccagcagctaatgggcgggcagacccaagagaagctgcccccgctcaccctcctcaagttgggcaaccaggagtccagtggccatattggcctgaagaaggccccaagagactgcaggggagccccaaccccagagcagacccgcagattggcccaggccatgatggccttcaccacagacctgttctccctggtggcccaaaggtccaccagccccaacctaatcctgtcgcctctgagtgtggccctggcactgtctcacctggcactaggtgctcagaaccagacgctgcggaggttagagcaggtgctgcatgtagactctgggccctgcctcccccacctgctgagccgcctttgccaggacctgggccctggggcattccgattggctgctagaatgtacctgcagaaaggatttcccatcaaagaggacttcctgaaacaatcagaacagctctttggtgccaagcccatgagcctgaccggaaggaaaggggatgatctgctaaacatcaaccaatgggtgaaggaggccacagaggggaagattgaggatttcctctcagagctgccagatgacacagtgttgcttctgctcaatgccatccacttccagggtttctggaggagcaagtttgatccaagcctcacccagagagacagtttccacctgaacgagcagttcacggtgccagtggacatgatgcacgcccgcacgtaccccctgcgctggttcctgctggagcagcctgagatacaggtggctcatttcccctttaagaacaacatgagctttgtggtcattatgcccacccactttgagtggaacgtgtcccaggtgctggccaacctgagctgggacatcctgcaccagcccttactgcgagagaaacccaccaaggtccggctgcctaagctgcacctgaactaccagctggacttggtggccaccctcagccggctgggcctgcaggagctgttccaggccccagacctgcgcgggatctccgaccagcgcctggtggtgaccagcgtgcagcaccagtctgctctggagctcagtgaggctggtgtggaggcggccgcggccacgggcacggccatgtcccgaatgtctctctcctccttcagcgtcaaccgccccttcctcttcttcatcctcgaggacacaacaagcctgcccctgtttgtgggcagtgtgaagaaccccaaccctagtgcgccatgggagcgcaaggagcagcaggattcccccgatgacagggactacttccagaaccggaaagcctttccccgcggagacaagcccttcgggcctgacttgaaacttgcgcctccctcagaggaggattacccccaacttcatagccccaagtga

SEQ ID NO: 6 - protein, 555 aa, Canis lupus
MGWLEPEQSVGSTTVGPEGHCVQQQGAYRGQQQGSPAHPTKPAETSGIHRPVYPCGQDQTKKRNMALLRGLLVISLSCLQGSGAVFPPASAMEPLDQQLMGGQTQEKLPPLTLLKLGNQESSGHIGLKKAPRDCRGAPTPEQTRRLAQAMMAFTTDLFSLVAQRSTSPNLILSPLSVALALSHLALGAQNQTLRRLEQVLHVDSGPCLPHLLSRLCQDLGPGAFRLAARMYLQKGFPIKEDFLKQSEQLFGAKPMSLTGRKGDDLLNINQWVKEATEGKIEDFLSELPDDTVLLLLNAIHFQGFWRSKFDPSLTQRDSFHLNEQFTVPVDMMHARTYPLRWFLLEQPEIQVAHFPFKNNMSFVVIMPTHFEWNVSQVLANLSWDILHQPLLREKPTKVRLPKLHLNYQLDLVATLSRLGLQELFQAPDLRGISDQRLVVTSVQHQSALELSEAGVEAAAATGTAMSRMSLSSFSVNRPFLFFILEDTTSLPLFVGSVKNPNPSAPWERKEQQDSPDDRDYFQNRKAFPRGDKPFGPDLKLAPPSEEDYPQLHSPK

SEQ ID NO: 7 - DNA, 18 bp, Artificial Sequence
  PCR primer
acgctgcggaggttagag

SEQ ID NO: 8 - DNA, 18 bp, Artificial Sequence
  PCR primer
cccaggtcctggcaaagg

SEQ ID NO: 9 - DNA, 17 bp, Artificial Sequence
  probe sequence
ccagagtctgcatgcag

SEQ ID NO: 10 - DNA, 17 bp, Artificial Sequence
  probe sequence
ccagagtctacatgcag

SEQ ID NO: 11 - DNA, 15 bp, Artificial Sequence
  PCR primer
cctcagcggggctgg

SEQ ID NO: 12 - DNA, 19 bp, Artificial Sequence
  PCR primer
gggcttgtttccgagcggg

SEQ ID NO: 13 - DNA, 18 bp, Artificial Sequence
  PCR primer
acgctgcggaggttagag

SEQ ID NO: 14 - DNA, 18 bp, Artificial Sequence
  PCR primer
cccaggtcctggcaaagg

SEQ ID NO: 15 - DNA, 17 bp, Artificial Sequence
  PCR primer
ccagagtctgcatgcag

SEQ ID NO: 16 - DNA, 17 bp, Artificial Sequence
  PCR primer
ccagagtctacatgcag